European Patent Specification EP 3 636 773 B1, published August 23, 2023. Title: N-cadherin and FGFR1 and/or FGFR4 for use in predicting the response of patients to a lung cancer treatment and method and kit based on said use. Applicant: Fundación Instituto de Investigación Hospital 12 de Octubre Servicio Andaluz de Salud Consejo Superior de Investigaciones Científicas. Application EP18836033. The sequence listing filed with the application follows.

SEQUENCE LISTING (6 sequences)

SEQ ID NO: 1 - DNA, 3873 bp, Homo sapiens
  Cadherin 2 (CDH2)
ctgctgccgctgctggcggccctgcttcaggcgtctgtagaggcttctggtgaaatcgcattatgcaagactggatttcctgaagatgtttacagtgcagtcttatcgaaggatgtgcatgaaggacagcctcttctcaatgtgaagtttagcaactgcaatggaaaaagaaaagtacaatatgagagcagtgagcctgcagattttaaggtggatgaagatggcatggtgtatgccgtgagaagctttccactctcttctgagcatgccaagttcctgatatatgcccaagacaaagagacccaggaaaagtggcaagtggcagtaaaattgagcctgaagccaaccttaactgaggagtcagtgaaggagtcagcagaagttgaagaaatagtgttcccaagacaattcagtaagcacagtggccacctacaaaggcagaagagagactgggtcatccctccaatcaacttgccagaaaactccaggggaccttttcctcaagagcttgtcaggatcaggtctgatagagataaaaacctttcactgcggtacagtgtaactgggccaggagctgaccagcctccaactggtatcttcattatcaaccccatctcgggtcagctgtcggtgacaaagcccctggatcgcgagcagatagcccggtttcatttgagggcacatgcagtagatattaatggaaatcaagtggagaaccccattgacattgtcatcaatgttattgacatgaatgacaacagacctgagttcttacaccaggtttggaatgggacagttcctgagggatcaaagcctggaacatatgtgatgaccgtaacagcaattgatgctgacgatcccaatgccctcaatgggatgttgaggtacagaatcgtgtctcaggctccaagcaccccttcacccaacatgtttacaatcaacaatgagactggtgacatcatcacagtggcagctggacttgatcgagaaaaagtgcaacagtatacgttaataattcaagctacagacatggaaggcaatcccacatatggcctttcaaacacagccacggccgtcatcacagtgacagatgtcaatgacaatcctccagagtttactgccatgacgttttatggtgaagttcctgagaacagggtagacatcatagtagctaatctaactgtgaccgataaggatcaaccccatacaccagcctggaacgcagtgtacagaatcagtggcggagatcctactggacggttcgccatccagaccgacccaaacagcaacgacgggttagtcaccgtggtcaaaccaatcgactttgaaacaaataggatgtttgtccttactgttgctgcagaaaatcaagtgccattagccaagggaattcagcacccgcctcagtcaactgcaaccgtgtctgttacagttattgacgtaaatgaaaacccttattttgcccccaatcctaagatcattcgccaagaagaagggcttcatgccggtaccatgttgacaacattcactgctcaggacccagatcgatatatgcagcaaaatattagatacactaaattatctgatcctgccaattggctaaaaatagatcctgtgaatggacaaataactacaattgctgttttggaccgagaatcaccaaatgtgaaaaacaatatatataatgctactttccttgcttctgacaatggaattcctcctatgagtggaacaggaacgctgcagatctatttacttgatattaatgacaatgcccctcaagtgttacctcaagaggcagagacttgcgaaactccagaccccaattcaattaatattacagcacttgattatgacattgatccaaatgctggaccatttgcttttgatcttcctttatctccagtgactattaagagaaattggaccatcactcggcttaatggtgattttgctcagcttaatttaaagataaaatttcttgaagctggtatctatgaagttcccatcataatcacagattcgggtaatcctcccaaatcaaatatttccatcctgcgcgtgaaggtttgccagtgtgactccaacggggactgcacagatgtggacaggattgtgggtgcggggcttggcaccggtgccatcattgccatcctgctctgcatcatcatcctgcttatccttgtgctgatgtttgtggtatggatgaaacgccgggataaagaacgccaggccaaacaacttttaattgatccagaagatgatgtaagagataatattttaaaatatgatgaagaaggtggaggagaagaagaccaggactatgacttgagccagctgcagcagcctgacactgtggagcctgatgccatcaagcctgtgggaatccgacgaatggatgaaagacccatccacgccgagccccagtatccggtccgatctgcagccccacaccctggagacattggggacttcattaatgagggccttaaagcggctgacaatgaccccacagctccaccatatgactccctgttagtgtttgactatgaaggcagtggctccactgctgggtccttgagctcccttaattcctcaagtagtggtggtgagcaggactatgattacctgaacgactgggggccacggttcaagaaacttgctgacatgtatggtggaggtgatgactgaacttcagggtgaacttggtttttggacaagtacaaacaatttcaactgatattcccaaaaagcattcagaagctaggctttaactttgtagtctactagcacagtgcttgctggaggctttggcataggctgcaaaccaatttgggctcagagggaatatcagtgatccatactgtttggaaaaacactgagctcagttacacttgaattttacagtacagaagcactgggattttatgtgcctttttgtacctttttcagattggaattagttttctgtttaaggctttaatggtactgatttctgaaacgataagtaaaagacaaaatattttgtggtgggagcagtaagttaaaccatgatatgcttcaacacgcttttgttacattgcatttgcttttattaaaatacaaaattaaacaaacaaaaaaactcatggagcgattttattatcttgggggatgagaccatgagattggaaaatgtacattacttctagttttagactttagtttgtttttttttttttcactaaaatcttaaaacttactcagctggttgcaaataaagggagttttcatatcaccaatttgtagcaaaattgaattttttcataaactagaatgttagacacattttggtcttaatccatgtacacttttttatttctgtatttttccacttcactgtaaaaatagtatgtgtacataatgttttattggcatagtctatggagaagtgcagaaacttcagaacatgtgtatgtattatttggactatggattcaggttttttgcatgtttatatctttcgttatggataaagtatttacaaaacagtgacatttgattcaattgttgagctgtagttagaatactcaatttttaatttttttaatttttttattttttattttctttttggtttggggagggagaaaagttcttagcacaaatgttttacataatttgtaccaaaaaaaaaaaaaaaggaaaggaaagaaaggggtggcctgacactggtggcactactaagtgtgtgtttttttaaaaaaaaaatggaaaaaaaaaagcttttaaactggagagacttctgacaacagctttgcctctgtattgtgtaccagaatataaatgatacacctctgaccccagcgttctgaataaaatgctaattttgga

SEQ ID NO: 2 - DNA, 2466 bp, Homo sapiens
  Fibroblast Growth Factor Receptor 1 (FGFR1) ORF, variant 1
atgtggagctggaagtgcctcctcttctgggctgtgctggtcacagccacactctgcaccgctaggccgtccccgaccttgcctgaacaagcccagccctggggagcccctgtggaagtggagtccttcctggtccaccccggtgacctgctgcagcttcgctgtcggctgcgggacgatgtgcagagcatcaactggctgcgggacggggtgcagctggcggaaagcaaccgcacccgcatcacaggggaggaggtggaggtgcaggactccgtgcccgcagactccggcctctatgcttgcgtaaccagcagcccctcgggcagtgacaccacctacttctccgtcaatgtttcagatgctctcccctcctcggaggatgatgatgatgatgatgactcctcttcagaggagaaagaaacagataacaccaaaccaaaccgtatgcccgtagctccatattggacatccccagaaaagatggaaaagaaattgcatgcagtgccggctgccaagacagtgaagttcaaatgcccttccagtgggaccccaaaccccacactgcgctggttgaaaaatggcaaagaattcaaacctgaccacagaattggaggctacaaggtccgttatgccacctggagcatcataatggactctgtggtgccctctgacaagggcaactacacctgcattgtggagaatgagtacggcagcatcaaccacacataccagctggatgtcgtggagcggtcccctcaccggcccatcctgcaagcagggttgcccgccaacaaaacagtggccctgggtagcaacgtggagttcatgtgtaaggtgtacagtgacccgcagccgcacatccagtggctaaagcacatcgaggtgaatgggagcaagattggcccagacaacctgccttatgtccagatcttgaagactgctggagttaataccaccgacaaagagatggaggtgcttcacttaagaaatgtctcctttgaggacgcaggggagtatacgtgcttggcgggtaactctatcggactctcccatcactctgcatggttgaccgttctggaagccctggaagagaggccggcagtgatgacctcgcccctgtacctggagatcatcatctattgcacaggggccttcctcatctcctgcatggtggggtcggtcatcgtctacaagatgaagagtggtaccaagaagagtgacttccacagccagatggctgtgcacaagctggccaagagcatccctctgcgcagacaggtaacagtgtctgctgactccagtgcatccatgaactctggggttcttctggttcggccatcacggctctcctccagtgggactcccatgctagcaggggtctctgagtatgagcttcccgaagaccctcgctgggagctgcctcgggacagactggtcttaggcaaacccctgggagagggctgctttgggcaggtggtgttggcagaggctatcgggctggacaaggacaaacccaaccgtgtgaccaaagtggctgtgaagatgttgaagtcggacgcaacagagaaagacttgtcagacctgatctcagaaatggagatgatgaagatgatcgggaagcataagaatatcatcaacctgctgggggcctgcacgcaggatggtcccttgtatgtcatcgtggagtatgcctccaagggcaacctgcgggagtacctgcaggcccggaggcccccagggctggaatactgctacaaccccagccacaacccagaggagcagctctcctccaaggacctggtgtcctgcgcctaccaggtggcccgaggcatggagtatctggcctccaagaagtgcatacaccgagacctggcagccaggaatgtcctggtgacagaggacaatgtgatgaagatagcagactttggcctcgcacgggacattcaccacatcgactactataaaaagacaaccaacggccgactgcctgtgaagtggatggcacccgaggcattatttgaccggatctacacccaccagagtgatgtgtggtctttcggggtgctcctgtgggagatcttcactctgggcggctccccataccccggtgtgcctgtggaggaacttttcaagctgctgaaggagggtcaccgcatggacaagcccagtaactgcaccaacgagctgtacatgatgatgcgggactgctggcatgcagtgccctcacagagacccaccttcaagcagctggtggaagacctggaccgcatcgtggccttgacctccaaccaggagtacctggacctgtccatgcccctggaccagtactcccccagctttcccgacacccggagctctacgtgctcctcaggggaggattccgtcttctctcatgagccgctgcccgaggagccctgcctgccccgacacccagcccagcttgccaatggcggactcaaacgccgc

SEQ ID NO: 3 - DNA, 2406 bp, Homo sapiens
  Fibroblast Growth Factor Receptor 4 (FGFR4) ORF, variant 1
atgcggctgctgctggccctgttgggggtcctgctgagtgtgcctgggcctccagtcttgtccctggaggcctctgaggaagtggagcttgagccctgcctggctcccagcctggagcagcaagagcaggagctgacagtagcccttgggcagcctgtgcgtctgtgctgtgggcgggctgagcgtggtggccactggtacaaggagggcagtcgcctggcacctgctggccgtgtacggggctggaggggccgcctagagattgccagcttcctacctgaggatgctggccgctacctctgcctggcacgaggctccatgatcgtcctgcagaatctcaccttgattacaggtgactccttgacctccagcaacgatgatgaggaccccaagtcccatagggacccctcgaataggcacagttacccccagcaagcaccctactggacacacccccagcgcatggagaagaaactgcatgcagtacctgcggggaacaccgtcaagttccgctgtccagctgcaggcaaccccacgcccaccatccgctggcttaaggatggacaggcctttcatggggagaaccgcattggaggcattcggctgcgccatcagcactggagtctcgtgatggagagcgtggtgccctcggaccgcggcacatacacctgcctggtagagaacgctgtgggcagcatccgctataactacctgctagatgtgctggagcggtccccgcaccggcccatcctgcaggccgggctcccggccaacaccacagccgtggtgggcagcgacgtggagctgctgtgcaaggtgtacagcgatgcccagccccacatccagtggctgaagcacatcgtcatcaacggcagcagcttcggagccgacggtttcccctatgtgcaagtcctaaagactgcagacatcaatagctcagaggtggaggtcctgtacctgcggaacgtgtcagccgaggacgcaggcgagtacacctgcctcgcaggcaattccatcggcctctcctaccagtctgcctggctcacggtgctgccagaggaggaccccacatggaccgcagcagcgcccgaggccaggtatacggacatcatcctgtacgcgtcgggctccctggccttggctgtgctcctgctgctggccgggctgtatcgagggcaggcgctccacggccggcacccccgcccgcccgccactgtgcagaagctctcccgcttccctctggcccgacagttctccctggagtcaggctcttccggcaagtcaagctcatccctggtacgaggcgtgcgtctctcctccagcggccccgccttgctcgccggcctcgtgagtctagatctacctctcgacccactatgggagttcccccgggacaggctggtgcttgggaagcccctaggcgagggctgctttggccaggtagtacgtgcagaggcctttggcatggaccctgcccggcctgaccaagccagcactgtggccgtcaagatgctcaaagacaacgcctctgacaaggacctggccgacctggtctcggagatggaggtgatgaagctgatcggccgacacaagaacatcatcaacctgcttggtgtctgcacccaggaagggcccctgtacgtgatcgtggagtgcgccgccaagggaaacctgcgggagttcctgcgggcccggcgccccccaggccccgacctcagccccgacggtcctcggagcagtgaggggccgctctccttcccagtcctggtctcctgcgcctaccaggtggcccgaggcatgcagtatctggagtcccggaagtgtatccaccgggacctggctgcccgcaatgtgctggtgactgaggacaatgtgatgaagattgctgactttgggctggcccgcggcgtccaccacattgactactataagaaaaccagcaacggccgcctgcctgtgaagtggatggcgcccgaggccttgtttgaccgggtgtacacacaccagagtgacgtgtggtcttttgggatcctgctatgggagatcttcaccctcgggggctccccgtatcctggcatcccggtggaggagctgttctcgctgctgcgggagggacatcggatggaccgacccccacactgccccccagagctgtacgggctgatgcgtgagtgctggcacgcagcgccctcccagaggcctaccttcaagcagctggtggaggcgctggacaaggtcctgctggccgtctctgaggagtacctcgacctccgcctgaccttcggaccctattccccctctggtggggacgccagcagcacctgctcctccagcgattctgtcttcagccacgaccccctgccattgggatccagctccttccccttcgggtctggggtgcagaca

SEQ ID NO: 4 - protein, 906 aa, Homo sapiens
  N-cadherin (NCBI: NP_001783.2)
MCRIAGALRTLLPLLAALLQASVEASGEIALCKTGFPEDVYSAVLSKDVHEGQPLLNVKFSNCNGKRKVQYESSEPADFKVDEDGMVYAVRSFPLSSEHAKFLIYAQDKETQEKWQVAVKLSLKPTLTEESVKESAEVEEIVFPRQFSKHSGHLQRQKRDWVIPPINLPENSRGPFPQELVRIRSDRDKNLSLRYSVTGPGADQPPTGIFIINPISGQLSVTKPLDREQIARFHLRAHAVDINGNQVENPIDIVINVIDMNDNRPEFLHQVWNGTVPEGSKPGTYVMTVTAIDADDPNALNGMLRYRIVSQAPSTPSPNMFTINNETGDIITVAAGLDREKVQQYTLIIQATDMEGNPTYGLSNTATAVITVTDVNDNPPEFTAMTFYGEVPENRVDIIVANLTVTDKDQPHTPAWNAVYRISGGDPTGRFAIQTDPNSNDGLVTVVKPIDFETNRMFVLTVAAENQVPLAKGIQHPPQSTATVSVTVIDVNENPYFAPNPKIIRQEEGLHAGTMLTTFTAQDPDRYMQQNIRYTKLSDPANWLKIDPVNGQITTIAVLDRESPNVKNNIYNATFLASDNGIPPMSGTGTLQIYLLDINDNAPQVLPQEAETCETPDPNSINITALDYDIDPNAGPFAFDLPLSPVTIKRNWTITRLNGDFAQLNLKIKFLEAGIYEVPIIITDSGNPPKSNISILRVKVCQCDSNGDCTDVDRIVGAGLGTGAIIAILLCIIILLILVLMFVVWMKRRDKERQAKQLLIDPEDDVRDNILKYDEEGGGEEDQDYDLSQLQQPDTVEPDAIKPVGIRRMDERPIHAEPQYPVRSAAPHPGDIGDFINEGLKAADNDPTAPPYDSLLVFDYEGSGSTAGSLSSLNSSSSGGEQDYDYLNDWGPRFKKLADMYGGGDD

SEQ ID NO: 5 - protein, 822 aa, Homo sapiens [sequence omitted]

SEQ ID NO: 6 - protein, 802 aa, Homo sapiens
  Fibroblast growth factor receptor 4 (FGFR4). NCBI: NP_002002.3
MRLLLALLGVLLSVPGPPVLSLEASEEVELEPCLAPSLEQQEQELTVALGQPVRLCCGRAERGGHWYKEGSRLAPAGRVRGWRGRLEIASFLPEDAGRYLCLARGSMIVLQNLTLITGDSLTSSNDDEDPKSHRDPSNRHSYPQQAPYWTHPQRMEKKLHAVPAGNTVKFRCPAAGNPTPTIRWLKDGQAFHGENRIGGIRLRHQHWSLVMESVVPSDRGTYTCLVENAVGSIRYNYLLDVLERSPHRPILQAGLPANTTAVVGSDVELLCKVYSDAQPHIQWLKHIVINGSSFGADGFPYVQVLKTADINSSEVEVLYLRNVSAEDAGEYTCLAGNSIGLSYQSAWLTVLPEEDPTWTAAAPEARYTDIILYASGSLALAVLLLLAGLYRGQALHGRHPRPPATVQKLSRFPLARQFSLESGSSGKSSSSLVRGVRLSSSGPALLAGLVSLDLPLDPLWEFPRDRLVLGKPLGEGCFGQVVRAEAFGMDPARPDQASTVAVKMLKDNASDKDLADLVSEMEVMKLIGRHKNIINLLGVCTQEGPLYVIVECAAKGNLREFLRARRPPGPDLSPDGPRSSEGPLSFPVLVSCAYQVARGMQYLESRKCIHRDLAARNVLVTEDNVMKIADFGLARGVHHIDYYKKTSNGRLPVKWMAPEALFDRVYTHQSDVWSFGILLWEIFTLGGSPYPGIPVEELFSLLREGHRMDRPPHCPPELYGLMRECWHAAPSQRPTFKQLVEALDKVLLAVSEEYLDLRLTFGPYSPSGGDASSTCSSSDSVFSHDPLPLGSSSFPFGSGVQT